European Patent Application EP 4 692 346 A1, published February 11, 2026. Title: crRNA with modified nucleotide. Applicant: Kyoto University. The sequence listing filed with the application follows.

SEQUENCE LISTING (193 sequences)

SEQ ID NO: 1 - RNA, 16 nt, Escherichia coli
  source 1..16: mol_type = transcribed RNA
ccccgcgccagcgggg

SEQ ID NO: 2 - DNA, 46 bp, synthetic construct
  misc_feature 1..46: note = PCR Primer
  source 1..46: mol_type = other DNA
gaaattaatacgactcactataggatgtgttgtttgtgtgatacta

SEQ ID NO: 3 - DNA, 18 bp, synthetic construct
  misc_feature 1..18: note = PCR Primer
  source 1..18: mol_type = other DNA
cccgggctgcaggaattc

SEQ ID NO: 4 - DNA, 32 bp, Homo sapiens
  source 1..32: mol_type = genomic DNA
gccacggagcgagacatctcggcccgaatgct

SEQ ID NO: 5 - DNA, 32 bp, Homo sapiens
  source 1..32: mol_type = genomic DNA
agagagtagcgcgagcacagctaaggccacgg

SEQ ID NO: 6 - DNA, 32 bp, Homo sapiens
  source 1..32: mol_type = genomic DNA
gctgggactccccaatccatacaccgccttcg

SEQ ID NO: 7 - DNA, 32 bp, Homo sapiens
  source 1..32: mol_type = genomic DNA
ccaatcagtgtcgtcgcggtcgctgttctaaa

SEQ ID NO: 8 - DNA, 32 bp, Homo sapiens
  source 1..32: mol_type = genomic DNA
tgaaggcccactcacagactgaccgagagaac

SEQ ID NO: 9 - DNA, 32 bp, Homo sapiens
  source 1..32: mol_type = genomic DNA
gcccactcacagactgaccgagagaacctgcg

SEQ ID NO: 10 - DNA, 32 bp, Homo sapiens
  source 1..32: mol_type = genomic DNA
gattacatcgccctgaaagaggacctgcgctc

SEQ ID NO: 11 - DNA, 32 bp, Homo sapiens
  source 1..32: mol_type = genomic DNA
tgggaggcggcccatgtggcggagcagcagag

SEQ ID NO: 12 - DNA, 32 bp, Homo sapiens
  source 1..32: mol_type = genomic DNA
gagacgctgcagcgcacgggtaccaggggcca

SEQ ID NO: 13 - DNA, 32 bp, Homo sapiens
  source 1..32: mol_type = genomic DNA
cgcccgtccgaccccacgtcgcagccaaacat

SEQ ID NO: 14 - DNA, 32 bp, Homo sapiens
  source 1..32: mol_type = genomic DNA
aggacctgcgctcttggaccgcggcggacatg

SEQ ID NO: 15 - DNA, 32 bp, Homo sapiens
  source 1..32: mol_type = genomic DNA
aaactgcggagttggggaatccccaaggctgg

SEQ ID NO: 16 - DNA, 32 bp, Homo sapiens
  source 1..32: mol_type = genomic DNA
atggccacatgcatgctggtggagtgtcccat

SEQ ID NO: 17 - DNA, 32 bp, Homo sapiens
  source 1..32: mol_type = genomic DNA
attatcccaggtgcctgtgtccaggctggtgt

SEQ ID NO: 18 - DNA, 32 bp, Homo sapiens
  source 1..32: mol_type = genomic DNA
tcgctgttccctcctcagggaatagaagatta

SEQ ID NO: 19 - DNA, 32 bp, Homo sapiens
  source 1..32: mol_type = genomic DNA
gctctcggagcctgagaccctgagagccccgc

SEQ ID NO: 20 - DNA, 32 bp, Homo sapiens
  source 1..32: mol_type = genomic DNA
aggaggaaaatgggatcagcgctagaatgtcg

SEQ ID NO: 21 - DNA, 32 bp, Homo sapiens
  source 1..32: mol_type = genomic DNA
agcagagatacacatgccatgtacagcatgag

SEQ ID NO: 22 - DNA, 32 bp, Homo sapiens
  source 1..32: mol_type = genomic DNA
gaccctacataggttgggagagggagaaaaga

SEQ ID NO: 23 - DNA, 32 bp, Homo sapiens
  source 1..32: mol_type = genomic DNA
aaggaccctacataggttgggagagggagaaa

SEQ ID NO: 24 - DNA, 32 bp, Homo sapiens
  source 1..32: mol_type = genomic DNA
gggtgaagggtggggtctgagatttcttgtct

SEQ ID NO: 25 - DNA, 32 bp, Homo sapiens; identical to SEQ ID NO: 17
  source 1..32: mol_type = genomic DNA

SEQ ID NO: 26 - DNA, 32 bp, Homo sapiens
  source 1..32: mol_type = genomic DNA
acgatccctcgaatactgatgactggttccct

SEQ ID NO: 27 - DNA, 32 bp, Homo sapiens
  source 1..32: mol_type = genomic DNA
ggataaaatctctgacggaatgacggaaagac

SEQ ID NO: 28 - DNA, 32 bp, Homo sapiens
  source 1..32: mol_type = genomic DNA
gaggggagacaattgggaccaacactagaata

SEQ ID NO: 29 - DNA, 32 bp, Homo sapiens
  source 1..32: mol_type = genomic DNA
tgaaactcgtgggagtggggaatccccaacgc

SEQ ID NO: 30 - DNA, 32 bp, Homo sapiens
  source 1..32: mol_type = genomic DNA
aagtgaaactcgtgggagtggggaatccccaa

SEQ ID NO: 31 - DNA, 32 bp, Homo sapiens
  source 1..32: mol_type = genomic DNA
gacccgacataggttgggagaagaagtgaaac

SEQ ID NO: 32 - DNA, 32 bp, Homo sapiens
  source 1..32: mol_type = genomic DNA
aaggacccgacataggttgggagaagaagtga

SEQ ID NO: 33 - DNA, 32 bp, Homo sapiens
  source 1..32: mol_type = genomic DNA
attacatcgccctgaacgaggacctgagctcc

SEQ ID NO: 34 - DNA, 32 bp, Homo sapiens
  source 1..32: mol_type = genomic DNA
cgcctgaattttctgactcttcccatcagacc

SEQ ID NO: 35 - DNA, 32 bp, Homo sapiens
  source 1..32: mol_type = genomic DNA
gagggggatgaggggtcatatctcttctcagg

SEQ ID NO: 36 - DNA, 32 bp, Homo sapiens
  source 1..32: mol_type = genomic DNA
ggatgacgtctctgaggaaatggaggggaaga

SEQ ID NO: 37 - DNA, 32 bp, Homo sapiens
  source 1..32: mol_type = genomic DNA
tccctgttccccgctcagagactcgaactttc

SEQ ID NO: 38 - DNA, 32 bp, Homo sapiens
  source 1..32: mol_type = genomic DNA
agctcaggtagggaaggggtgaggggtggggt

SEQ ID NO: 39 - DNA, 32 bp, Homo sapiens
  source 1..32: mol_type = genomic DNA
gccgcttccgaaccgcccacgggcctccgctt

SEQ ID NO: 40 - DNA, 32 bp, Homo sapiens
  source 1..32: mol_type = genomic DNA
gccgcttccgaatcgcccacgggcctccgctt

SEQ ID NO: 41 - DNA, 32 bp, Homo sapiens
  source 1..32: mol_type = genomic DNA
ccgcttccgaaccgcccacgggcctccgcttc

SEQ ID NO: 42 - DNA, 30 bp, Homo sapiens
  source 1..30: mol_type = genomic DNA
gccgcttccgaaccgcccacgggcctccgc

SEQ ID NO: 43 - DNA, 28 bp, Homo sapiens
  source 1..28: mol_type = genomic DNA
gccgcttccgaaccgcccacgggcctcc

SEQ ID NO: 44 - DNA, 26 bp, Homo sapiens
  source 1..26: mol_type = genomic DNA
gccgcttccgaaccgcccacgggcct

SEQ ID NO: 45 - DNA, 32 bp, Homo sapiens
  source 1..32: mol_type = genomic DNA
gccgcttccgaaccgcccacgggcctccgctg

SEQ ID NO: 46 - DNA, 32 bp, Homo sapiens
  source 1..32: mol_type = genomic DNA
gccgcttccgaaccgcccacgggcctccgcgt

SEQ ID NO: 47 - DNA, 32 bp, Homo sapiens
  source 1..32: mol_type = genomic DNA
gccgcttccgaaccgcccacgggcctccactt

SEQ ID NO: 48 - DNA, 32 bp, Homo sapiens
  source 1..32: mol_type = genomic DNA
cgggtggcaaggggcgggtggagcgcggggcg

SEQ ID NO: 49 - DNA, 32 bp, Homo sapiens
  source 1..32: mol_type = genomic DNA
cgcagctaagcgggtggcaaggggcgggtgga

SEQ ID NO: 50 - DNA, 32 bp, Homo sapiens
  source 1..32: mol_type = genomic DNA
tgcgcagctaagcgggtggcaaggggcgggtg

SEQ ID NO: 51 - DNA, 32 bp, Homo sapiens
  source 1..32: mol_type = genomic DNA
ggatgccaagggttgccaccggcccgcatccc

SEQ ID NO: 52 - DNA, 32 bp, Homo sapiens
  source 1..32: mol_type = genomic DNA
gggatgccaagggttgccaccggcccgcatcc

SEQ ID NO: 53 - DNA, 32 bp, Homo sapiens
  source 1..32: mol_type = genomic DNA
tcctcggacatctcccgggaccagctcacaat

SEQ ID NO: 54 - DNA, 32 bp, Homo sapiens
  source 1..32: mol_type = genomic DNA
gtggtcccagctcggggacacaggatccctgg

SEQ ID NO: 55 - DNA, 32 bp, Homo sapiens
  source 1..32: mol_type = genomic DNA
ctgacagtagaccccagtacatgcttcctaaa

SEQ ID NO: 56 - DNA, 32 bp, Homo sapiens
  source 1..32: mol_type = genomic DNA
tcttggtgagaatcatattctgtagtacaagg

SEQ ID NO: 57 - DNA, 32 bp, Homo sapiens
  source 1..32: mol_type = genomic DNA
actccatctcaaatacatacatacatacgtac

SEQ ID NO: 58 - DNA, 32 bp, Homo sapiens
  source 1..32: mol_type = genomic DNA
gaaactgagacaaaggggttaaataccagctc

SEQ ID NO: 59 - DNA, 32 bp, Homo sapiens
  source 1..32: mol_type = genomic DNA
attgtaaaaggaagtcccttcatgtacaagga

SEQ ID NO: 60 - DNA, 32 bp, Homo sapiens
  source 1..32: mol_type = genomic DNA
cttattatttattaatgagtcaaacaggcctt

SEQ ID NO: 61 - DNA, 32 bp, Homo sapiens
  source 1..32: mol_type = genomic DNA
ttcatgcctttccccaggcagccctcattcag

SEQ ID NO: 62 - DNA, 32 bp, Homo sapiens
  source 1..32: mol_type = genomic DNA
ttggcatttatgcaatgccatgttcaaatgaa

SEQ ID NO: 63 - DNA, 32 bp, Homo sapiens
  source 1..32: mol_type = genomic DNA
acccatctgactagacgctgtgcatattcttt

SEQ ID NO: 64 - DNA, 32 bp, Homo sapiens
  source 1..32: mol_type = genomic DNA
atcacttcaaaattggtatacgtatttatgta

SEQ ID NO: 65 - DNA, 32 bp, Homo sapiens
  source 1..32: mol_type = genomic DNA
ccttgtatccttattatacctctcttgatctc

SEQ ID NO: 66 - DNA, 32 bp, Homo sapiens
  source 1..32: mol_type = genomic DNA
cctgaatctgcggtggcaggaggtctgcaaac

SEQ ID NO: 67 - DNA, 32 bp, Homo sapiens
  source 1..32: mol_type = genomic DNA
ctcaagcagacaaatctccagtggataaaggt

SEQ ID NO: 68 - DNA, 32 bp, Homo sapiens
  source 1..32: mol_type = genomic DNA
acaaaatattacttgttaaagtgtggtaagga

SEQ ID NO: 69 - DNA, 24 bp, synthetic construct
  misc_feature 1..24: note = PCR Primer
  source 1..24: mol_type = other DNA
gagtgtggcttggacttaatgagg

SEQ ID NO: 70 - DNA, 22 bp, synthetic construct
  misc_feature 1..22: note = PCR Primer
  source 1..22: mol_type = other DNA
agctcagtgcaccatgaagttg

SEQ ID NO: 71 - DNA, 25 bp, synthetic construct
  misc_feature 1..25: note = PCR Primer
  source 1..25: mol_type = other DNA
ccctggctcacacgtgtactgacac

SEQ ID NO: 72 - DNA, 20 bp, synthetic construct
  misc_feature 1..20: note = PCR Primer
  source 1..20: mol_type = other DNA
aagcggaggcccgtggacgg

SEQ ID NO: 73 - DNA, 20 bp, synthetic construct
  misc_feature 1..20: note = PCR Primer
  source 1..20: mol_type = other DNA
aagcggaggcccgtggacga

SEQ ID NO: 74 - DNA, 28 bp, synthetic construct
  misc_feature 1..28: note = PCR Primer
  source 1..28: mol_type = other DNA
ggccagaagttctggttctccacccgag

SEQ ID NO: 75 - DNA, 20 bp, synthetic construct
  misc_feature 1..20: note = PCR Primer
  source 1..20: mol_type = other DNA
cgggcgcctgagattgggag

SEQ ID NO: 76 - DNA, 24 bp, synthetic construct
  misc_feature 1..24: note = PCR Primer
  source 1..24: mol_type = other DNA
cgggccggtggcaacccttgacat

SEQ ID NO: 77 - DNA, 20 bp, synthetic construct
  misc_feature 1..20: note = PCR Primer
  source 1..20: mol_type = other DNA
accagttgctgacctgcgtg

SEQ ID NO: 78 - DNA, 22 bp, synthetic construct
  misc_feature 1..22: note = PCR Primer
  source 1..22: mol_type = other DNA
cgcgggcgcctgagattgggag

SEQ ID NO: 79 - DNA, 22 bp, synthetic construct
  misc_feature 1..22: note = PCR Primer
  source 1..22: mol_type = other DNA
cgcgggcgcctgagattgtaag

SEQ ID NO: 80 - DNA, 21 bp, synthetic construct
  misc_feature 1..21: note = PCR Primer
  source 1..21: mol_type = other DNA
acatctgatgtgtgcccatgc

SEQ ID NO: 81 - DNA, 25 bp, synthetic construct
  misc_feature 1..25: note = PCR Primer
  source 1..25: mol_type = other DNA
cgcaaatgttgaggttttcagaggc

SEQ ID NO: 82 - DNA, 28 bp, synthetic construct
  misc_feature 1..28: note = PCR Primer
  source 1..28: mol_type = other DNA
ggatttggctgaaaatcacattgtctcg

SEQ ID NO: 83 - DNA, 29 bp, synthetic construct
  misc_feature 1..29: note = PCR Primer
  source 1..29: mol_type = other DNA
gaggctataaaagccaagaactgacaatg

SEQ ID NO: 84 - DNA, 27 bp, synthetic construct
  misc_feature 1..27: note = PCR Primer
  source 1..27: mol_type = other DNA
catttgccagtcagcctggtgttctgc

SEQ ID NO: 85 - DNA, 30 bp, synthetic construct
  misc_feature 1..30: note = PCR Primer
  source 1..30: mol_type = other DNA
ctatggtatacatctgatgtgtgcccatgc

SEQ ID NO: 86 - DNA, 27 bp, synthetic construct
  misc_feature 1..27: note = PCR Primer
  source 1..27: mol_type = other DNA
cttctggcctaccatttgttgatcacc

SEQ ID NO: 87 - DNA, 30 bp, synthetic construct
  misc_feature 1..30: note = PCR Primer
  source 1..30: mol_type = other DNA
cctaccatagctgatgggtaaaatgtaaac

SEQ ID NO: 88 - DNA, 33 bp, synthetic construct
  misc_feature 1..33: note = PCR Primer
  source 1..33: mol_type = other DNA
gaagcttgcagtttcttgagattagaaatagag

SEQ ID NO: 89 - DNA, 33 bp, synthetic construct
  misc_feature 1..33: note = PCR Primer
  source 1..33: mol_type = other DNA
gactggtgtctctattactaagcaatgactgtc

SEQ ID NO: 90 - DNA, 30 bp, synthetic construct
  misc_feature 1..30: note = PCR Primer
  source 1..30: mol_type = other DNA
gcaaatgcttactgaaaccttccatgcatc

SEQ ID NO: 91 - DNA, 22 bp, synthetic construct
  misc_feature 1..22: note = PCR Primer
  source 1..22: mol_type = other DNA
gactccatggtgatgatgagcc

SEQ ID NO: 92 - DNA, 24 bp, synthetic construct
  misc_feature 1..24: note = PCR Primer
  source 1..24: mol_type = other DNA
ctcctccgctcatccttttcactg

SEQ ID NO: 93 - DNA, 24 bp, synthetic construct
  misc_feature 1..24: note = PCR Primer
  source 1..24: mol_type = other DNA
caccacaggctttaacttctgccg

SEQ ID NO: 94 - DNA, 23 bp, synthetic construct
  misc_feature 1..23: note = PCR Primer
  source 1..23: mol_type = other DNA
ggttaagccactggacaaaaacg

SEQ ID NO: 95 - DNA, 23 bp, synthetic construct
  misc_feature 1..23: note = PCR Primer
  source 1..23: mol_type = other DNA
gagtagcctgatcgacactggac

SEQ ID NO: 96 - DNA, 21 bp, synthetic construct
  misc_feature 1..21: note = PCR Primer
  source 1..21: mol_type = other DNA
cctgaagtacaaggacgacgg

SEQ ID NO: 97 - DNA, 22 bp, synthetic construct
  misc_feature 1..22: note = PCR Primer
  source 1..22: mol_type = other DNA
cttcagaattaatccgtgcgcc

SEQ ID NO: 98 - DNA, 24 bp, synthetic construct
  misc_feature 1..24: note = PCR Primer
  source 1..24: mol_type = other DNA
cacacacaaaccaccgaaccaaag

SEQ ID NO: 99 - DNA, 25 bp, synthetic construct
  misc_feature 1..25: note = PCR Primer
  source 1..25: mol_type = other DNA
gtagacttagaatggaattctgggc

SEQ ID NO: 100 - DNA, 26 bp, synthetic construct
  misc_feature 1..26: note = PCR Primer
  source 1..26: mol_type = other DNA
gaatgggtcctggtgctgtgcttagc

SEQ ID NO: 101 - DNA, 20 bp, synthetic construct
  misc_feature 1..20: note = PCR Primer
  source 1..20: mol_type = other DNA
ccgcggtatctgttgttcgc

SEQ ID NO: 102 - DNA, 21 bp, synthetic construct
  misc_feature 1..21: note = ddPCR probe
  source 1..21: mol_type = other DNA
cccaaccccaggcagggcagc

SEQ ID NO: 103 - DNA, 20 bp, synthetic construct
  misc_feature 1..20: note = PCR Primer
  source 1..20: mol_type = other DNA
agctgagctggtatccaatg

SEQ ID NO: 104 - DNA, 20 bp, synthetic construct
  misc_feature 1..20: note = PCR Primer
  source 1..20: mol_type = other DNA
attcctgggtaagtcctggt

SEQ ID NO: 105 - DNA, 24 bp, synthetic construct
  misc_feature 1..24: note = ddPCR probe
  source 1..24: mol_type = other DNA
ccaccaccacgaaatggcggcacc

SEQ ID NO: 106 - DNA, 20 bp, synthetic construct
  misc_feature 1..20: note = PCR Primer
  source 1..20: mol_type = other DNA
gacttccaagatctctgccc

SEQ ID NO: 107 - DNA, 20 bp, synthetic construct
  misc_feature 1..20: note = PCR Primer
  source 1..20: mol_type = other DNA
taaacatgacaggcagaccc

SEQ ID NO: 108 - DNA, 20 bp, synthetic construct
  misc_feature 1..20: note = ddPCR probe
  source 1..20: mol_type = other DNA
ccacagggcccatgccgccc

SEQ ID NO: 109 - DNA, 20 bp, synthetic construct
  misc_feature 1..20: note = PCR Primer
  source 1..20: mol_type = other DNA
acacaggggataaatggcag

SEQ ID NO: 110 - DNA, 20 bp, synthetic construct
  misc_feature 1..20: note = PCR Primer
  source 1..20: mol_type = other DNA
gaaacaaccaggcaaagagc

SEQ ID NO: 111 - DNA, 21 bp, synthetic construct
  misc_feature 1..21: note = ddPCR probe
  source 1..21: mol_type = other DNA
ggcgtgagccaccgtgcctgc

SEQ ID NO: 112 - DNA, 20 bp, synthetic construct
  misc_feature 1..20: note = PCR Primer
  source 1..20: mol_type = other DNA
ttaactcttcacctggctgc

SEQ ID NO: 113 - DNA, 20 bp, synthetic construct
  misc_feature 1..20: note = PCR Primer
  source 1..20: mol_type = other DNA
ctgctcaccttgactttcca

SEQ ID NO: 114 - DNA, 25 bp, synthetic construct
  misc_feature 1..25: note = ddPCR probe
  source 1..25: mol_type = other DNA
tgtgccctgagtgcttctccctggc

SEQ ID NO: 115 - DNA, 20 bp, synthetic construct
  misc_feature 1..20: note = PCR Primer
  source 1..20: mol_type = other DNA
agcaggtcatttcagtagcc

SEQ ID NO: 116 - DNA, 20 bp, synthetic construct
  misc_feature 1..20: note = PCR Primer
  source 1..20: mol_type = other DNA
actaaggcatgctccaaagg

SEQ ID NO: 117 - DNA, 25 bp, synthetic construct
  misc_feature 1..25: note = ddPCR probe
  source 1..25: mol_type = other DNA
accccatcctgttggccacaaccca

SEQ ID NO: 118 - DNA, 20 bp, synthetic construct
  misc_feature 1..20: note = PCR Primer
  source 1..20: mol_type = other DNA
tctatgaggaaggactgcca

SEQ ID NO: 119 - DNA, 20 bp, synthetic construct
  misc_feature 1..20: note = PCR Primer
  source 1..20: mol_type = other DNA
ttgttctgtaccagggcttg

SEQ ID NO: 120 - DNA, 27 bp, synthetic construct
  misc_feature 1..27: note = ddPCR probe
  source 1..27: mol_type = other DNA
gtgagactctgtcccaccctcccacca

SEQ ID NO: 121 - DNA, 20 bp, synthetic construct
  misc_feature 1..20: note = PCR Primer
  source 1..20: mol_type = other DNA
tggggtagtccatggtagtt

SEQ ID NO: 122 - DNA, 20 bp, synthetic construct
  misc_feature 1..20: note = PCR Primer
  source 1..20: mol_type = other DNA
gagttgagatgcaccactgt

SEQ ID NO: 123 - DNA, 27 bp, synthetic construct
  misc_feature 1..27: note = ddPCR probe
  source 1..27: mol_type = other DNA
tccccagggaagccttctcatccagca

SEQ ID NO: 124 - DNA, 20 bp, synthetic construct
  misc_feature 1..20: note = PCR Primer
  source 1..20: mol_type = other DNA
tgctccacctgctactaaga

SEQ ID NO: 125 - DNA, 20 bp, synthetic construct
  misc_feature 1..20: note = PCR Primer
  source 1..20: mol_type = other DNA
gaggacaggtgtgattacgg

SEQ ID NO: 126 - DNA, 20 bp, synthetic construct
  misc_feature 1..20: note = ddPCR probe
  source 1..20: mol_type = other DNA
cctctggctcgcggcgtcgc

SEQ ID NO: 127 - DNA, 20 bp, synthetic construct
  misc_feature 1..20: note = PCR Primer
  source 1..20: mol_type = other DNA
ctcccactccatgaggtatt

SEQ ID NO: 128 - DNA, 20 bp, synthetic construct
  misc_feature 1..20: note = PCR Primer
  source 1..20: mol_type = other DNA
ccttcactttccctgtctcc

SEQ ID NO: 129 - DNA, 20 bp, synthetic construct
  misc_feature 1..20: note = ddPCR probe
  source 1..20: mol_type = other DNA
cctcggactcgcggcgtcgc

SEQ ID NO: 130 - DNA, 20 bp, synthetic construct
  misc_feature 1..20: note = PCR Primer
  source 1..20: mol_type = other DNA
atttctacaccgccatgtcc

SEQ ID NO: 131 - DNA, 20 bp, synthetic construct
  misc_feature 1..20: note = PCR Primer
  source 1..20: mol_type = other DNA
gcaggttctctcggtaagtc

SEQ ID NO: 132 - DNA, 18 bp, synthetic construct
  misc_feature 1..18: note = PCR Primer
  source 1..18: mol_type = other DNA
tgtgttttaggccagacc

SEQ ID NO: 133 - DNA, 18 bp, synthetic construct
  misc_feature 1..18: note = PCR Primer
  source 1..18: mol_type = other DNA
agcagtggtagtccagaa

SEQ ID NO: 134 - DNA, 26 bp, synthetic construct
  misc_feature 1..26: note = ddPCR probe
  source 1..26: mol_type = other DNA
agtcgttgtgtggctgactgctggca

SEQ ID NO: 135 - DNA, 21 bp, synthetic construct
  misc_feature 1..21: note = PCR Primer
  source 1..21: mol_type = other DNA
ggaactccaggatggcattgg

SEQ ID NO: 136 - DNA, 19 bp, synthetic construct
  misc_feature 1..19: note = PCR Primer
  source 1..19: mol_type = other DNA
gacagctgtttgcagacct

SEQ ID NO: 137 - DNA, 25 bp, synthetic construct
  misc_feature 1..25: note = ddPCR probe
  source 1..25: mol_type = other DNA
tgggaagcctgaatctgcggtggca

SEQ ID NO: 138 - DNA, 19 bp, synthetic construct
  misc_feature 1..19: note = PCR Primer
  source 1..19: mol_type = other DNA
ccccaggaagggcattaag

SEQ ID NO: 139 - DNA, 18 bp, synthetic construct
  misc_feature 1..18: note = PCR Primer
  source 1..18: mol_type = other DNA
agttcagatgttgtcccc

SEQ ID NO: 140 - DNA, 24 bp, synthetic construct
  misc_feature 1..24: note = ddPCR probe
  source 1..24: mol_type = other DNA
cccccatgaccccacacttcccgt

SEQ ID NO: 141 - DNA, 20 bp, synthetic construct
  misc_feature 1..20: note = PCR Primer
  source 1..20: mol_type = other DNA
ctgacttccctcttggtgac

SEQ ID NO: 142 - DNA, 20 bp, synthetic construct
  misc_feature 1..20: note = PCR Primer
  source 1..20: mol_type = other DNA
caggaatgagcatgtgacct

SEQ ID NO: 143 - DNA, 27 bp, synthetic construct
  misc_feature 1..27: note = ddPCR probe
  source 1..27: mol_type = other DNA
tggcctgaagccgtttcagaacccaca

SEQ ID NO: 144 - DNA, 18 bp, synthetic construct
  misc_feature 1..18: note = PCR Primer
  source 1..18: mol_type = other DNA
tgcagctttactccacac

SEQ ID NO: 145 - DNA, 20 bp, synthetic construct
  misc_feature 1..20: note = PCR Primer
  source 1..20: mol_type = other DNA
ggcagttcaagatttgctgg

SEQ ID NO: 146 - DNA, 26 bp, synthetic construct
  misc_feature 1..26: note = ddPCR probe
  source 1..26: mol_type = other DNA
cccaggaccctagcggaaagagcagc

SEQ ID NO: 147 - DNA, 20 bp, synthetic construct
  misc_feature 1..20: note = PCR Primer
  source 1..20: mol_type = other DNA
ctgttgctggatactttcgc

SEQ ID NO: 148 - DNA, 19 bp, synthetic construct
  misc_feature 1..19: note = PCR Primer
  source 1..19: mol_type = other DNA
cgactcactctcctctcat

SEQ ID NO: 149 - DNA, 26 bp, synthetic construct
  misc_feature 1..26: note = ddPCR probe
  source 1..26: mol_type = other DNA
cccaggaccctagcggaaagagcagc

SEQ ID NO: 150 - DNA, 20 bp, synthetic construct
  misc_feature 1..20: note = PCR Primer
  source 1..20: mol_type = other DNA
caatggctggaagctaagga

SEQ ID NO: 151 - DNA, 20 bp, synthetic construct
  misc_feature 1..20: note = PCR Primer
  source 1..20: mol_type = other DNA
tgtatagggaccctccttcc

SEQ ID NO: 152 - DNA, 27 bp, synthetic construct
  misc_feature 1..27: note = ddPCR probe
  source 1..27: mol_type = other DNA
agcaggtcttaggacaggccagagcca

SEQ ID NO: 153 - DNA, 20 bp, synthetic construct
  misc_feature 1..20: note = PCR Primer
  source 1..20: mol_type = other DNA
ggctgctttggaagaaactc

SEQ ID NO: 154 - DNA, 20 bp, synthetic construct
  misc_feature 1..20: note = PCR Primer
  source 1..20: mol_type = other DNA
cagctcttttactcccttgg

SEQ ID NO: 155 - DNA, 27 bp, synthetic construct
  misc_feature 1..27: note = ddPCR probe
  source 1..27: mol_type = other DNA
actgcaacagttccccctggacctgga

SEQ ID NO: 156 - DNA, 20 bp, synthetic construct
  misc_feature 1..20: note = PCR Primer
  source 1..20: mol_type = other DNA
cccagcttggtcaagcataa

SEQ ID NO: 157 - DNA, 20 bp, synthetic construct
  misc_feature 1..20: note = PCR Primer
  source 1..20: mol_type = other DNA
agactgcaactttaggccag

SEQ ID NO: 158 - DNA, 27 bp, synthetic construct
  misc_feature 1..27: note = ddPCR probe
  source 1..27: mol_type = other DNA
tcagtaacggtggagacctaggcggca

SEQ ID NO: 159 - DNA, 20 bp, synthetic construct
  misc_feature 1..20: note = PCR Primer
  source 1..20: mol_type = other DNA
tcaccacttcagcctctact

SEQ ID NO: 160 - DNA, 20 bp, synthetic construct
  misc_feature 1..20: note = PCR Primer
  source 1..20: mol_type = other DNA
aggacggtatgaaaagccac

SEQ ID NO: 161 - DNA, 24 bp, synthetic construct
  misc_feature 1..24: note = ddPCR probe
  source 1..24: mol_type = other DNA
accaacaccacgtcccacaccccc

SEQ ID NO: 162 - DNA, 20 bp, synthetic construct
  misc_feature 1..20: note = PCR Primer
  source 1..20: mol_type = other DNA
tggtaggaagatgagctggt

SEQ ID NO: 163 - DNA, 20 bp, synthetic construct
  misc_feature 1..20: note = PCR Primer
  source 1..20: mol_type = other DNA
agtatgggggatcctcttcc

SEQ ID NO: 164 - DNA, 26 bp, synthetic construct
  misc_feature 1..26: note = ddPCR probe
  source 1..26: mol_type = other DNA
ccccacatgtcaagggtggagccagg

SEQ ID NO: 165 - DNA, 20 bp, synthetic construct
  misc_feature 1..20: note = PCR Primer
  source 1..20: mol_type = other DNA
acgttgcctcaagttctctg

SEQ ID NO: 166 - DNA, 20 bp, synthetic construct
  misc_feature 1..20: note = PCR Primer
  source 1..20: mol_type = other DNA
agtgaaaaggatgagcggag

SEQ ID NO: 167 - DNA, 26 bp, synthetic construct
  misc_feature 1..26: note = ddPCR probe
  source 1..26: mol_type = other DNA
cccaggccccaatatacaccgagggc

SEQ ID NO: 168 - RNA, 90 nt, Escherichia coli
  misc_feature 30..61: note = n is a, c, g, or t
  source 1..90: mol_type = transcribed RNA
gtgttccccgcgccagcggggataaaccgnnnnnnnnnnnnnnnnnnnnnnnnnnnnnnnngtgttccccgcgccagcggggataaaccg

SEQ ID NO: 169 - RNA, 29 nt, Thermus thermophilus
  source 1..29: mol_type = transcribed RNA
gtagtccccacgcgtgtggggatggaccg

SEQ ID NO: 170 - RNA, 28 nt, Pseudomonas aeruginosa
  source 1..28: mol_type = transcribed RNA
gttcactgccgtataggcagctaagaaa

SEQ ID NO: 171 - RNA, 32 nt, Bacillus halodurans
  source 1..32: mol_type = transcribed RNA
gtcgcactcttcatgggtgcgtggattgaaat

SEQ ID NO: 172 - RNA, 24 nt, Sulfolobus solfataricus
  source 1..24: mol_type = transcribed RNA
gctaatctactatagaattgaaag

SEQ ID NO: 173 - RNA, 37 nt, Methanococcus maripaludis
  source 1..37: mol_type = transcribed RNA
ctaaaagaataacttgcaaaataacaagcattgaaag

SEQ ID NO: 174 - RNA, 30 nt, Pyrococcus furiosus
  source 1..30: mol_type = transcribed RNA
gttacaataagactaaaatagaattgaaag

SEQ ID NO: 175 - DNA, 30 bp, Homo sapiens
  source 1..30: mol_type = genomic DNA
cccctaacgcctgctcccatgttactcaag

SEQ ID NO: 176 - DNA, 30 bp, Homo sapiens
  source 1..30: mol_type = genomic DNA
ggtaaagagtgagatttctgatctctcttt

SEQ ID NO: 177 - DNA, 31 bp, Homo sapiens
  source 1..31: mol_type = genomic DNA
tgcctatgtttcctcataagcagcatacctt

SEQ ID NO: 178 - DNA, 30 bp, Homo sapiens
  source 1..30: mol_type = genomic DNA
ttcagatttaaatacaaggaggctcttaaa

SEQ ID NO: 179 - DNA, 30 bp, Homo sapiens
  source 1..30: mol_type = genomic DNA
ttcagatttaaatacaattccagaatcaaa

SEQ ID NO: 180 - DNA, 31 bp, Homo sapiens
  source 1..31: mol_type = genomic DNA
catctattaggagaggctcttaaagtttatt

SEQ ID NO: 181 - DNA, 40 bp, Homo sapiens
  source 1..40: mol_type = genomic DNA
ccgaggccgcttccgaaccgcccacgggcctccgcttctc

SEQ ID NO: 182 - DNA, 40 bp, Homo sapiens
  source 1..40: mol_type = genomic DNA
gagaagcggaggcccgtgggcggttcggaagcggcctcgg

SEQ ID NO: 183 - DNA, 35 bp, Homo sapiens
  misc_feature 9: note = n is a, c, g, or t
  misc_feature 15: note = n is a, c, g, or t
  misc_feature 21: note = n is a, c, g, or t
  misc_feature 27: note = n is a, c, g, or t
  misc_feature 33: note = n is a, c, g, or t
  source 1..35: mol_type = genomic DNA
gaggccgcntccganccgccnacgggnctccgntt

SEQ ID NO: 184 - DNA, 35 bp, Homo sapiens
  misc_feature 9: note = n is a, c, g, or t
  misc_feature 15: note = n is a, c, g, or t
  misc_feature 21: note = n is a, c, g, or t
  misc_feature 27: note = n is a, c, g, or t
  misc_feature 33: note = n is a, c, g, or t
  source 1..35: mol_type = genomic DNA
aggccgctnccgaancgcccncgggcntccgcntc

SEQ ID NO: 185 - DNA, 50 bp, Homo sapiens
  source 1..50: mol_type = genomic DNA
cggggccgggatgcgggccggtggcaacccttggcatcccctctcgtccg

SEQ ID NO: 186 - DNA, 50 bp, Homo sapiens
  source 1..50: mol_type = genomic DNA
cggacgagaggggatgccaagggttgccaccggcccgcatcccggccccg

SEQ ID NO: 187 - DNA, 35 bp, Homo sapiens
  misc_feature 9: note = n is a, c, g, or t
  misc_feature 15: note = n is a, c, g, or t
  misc_feature 21: note = n is a, c, g, or t
  misc_feature 27: note = n is a, c, g, or t
  misc_feature 33: note = n is a, c, g, or t
  source 1..35: mol_type = genomic DNA
aggggatgncaaggnttgccnccggcncgcatncc

SEQ ID NO: 188 - DNA, 35 bp, Homo sapiens
  misc_feature 9: note = n is a, c, g, or t
  misc_feature 15: note = n is a, c, g, or t
  misc_feature 21: note = n is a, c, g, or t
  misc_feature 27: note = n is a, c, g, or t
  misc_feature 33: note = n is a, c, g, or t
  source 1..35: mol_type = genomic DNA
gaggggatnccaagngttgcnaccggnccgcancc

SEQ ID NO: 189 - DNA, 57 bp, Homo sapiens
  source 1..57: mol_type = genomic DNA
ccgtcgcgccccgcgctccacccgccccttgccacccgcttagctgcgcatttgcgg

SEQ ID NO: 190 - DNA, 57 bp, Homo sapiens
  source 1..57: mol_type = genomic DNA
ccgcaaatgcgcagctaagcgggtggcaaggggcgggtggagcgcggggcgcgacgg

SEQ ID NO: 191 - DNA, 35 bp, Homo sapiens
  misc_feature 9: note = n is a, c, g, or t
  misc_feature 15: note = n is a, c, g, or t
  misc_feature 21: note = n is a, c, g, or t
  misc_feature 27: note = n is a, c, g, or t
  misc_feature 33: note = n is a, c, g, or t
  source 1..35: mol_type = genomic DNA
aagcgggtngcaagnggcggntggagngcgggncg

SEQ ID NO: 192 - DNA, 35 bp, Homo sapiens
  misc_feature 9: note = n is a, c, g, or t
  misc_feature 15: note = n is a, c, g, or t
  misc_feature 21: note = n is a, c, g, or t
  misc_feature 27: note = n is a, c, g, or t
  misc_feature 33: note = n is a, c, g, or t
  source 1..35: mol_type = genomic DNA
atgcgcagntaagcnggtggnaagggncgggtnga

SEQ ID NO: 193 - DNA, 35 bp, Homo sapiens
  misc_feature 9: note = n is a, c, g, or t
  misc_feature 15: note = n is a, c, g, or t
  misc_feature 21: note = n is a, c, g, or t
  misc_feature 27: note = n is a, c, g, or t
  misc_feature 33: note = n is a, c, g, or t
  source 1..35: mol_type = genomic DNA
aaatgcgcngctaancgggtngcaagnggcggntg